European Patent Specification EP 3 191 581 B9, published October 11, 2023. Title: Targeted Mutagenesis in Spirulina. Applicant: Matrix Genetics. The sequence listing filed with the application follows.

SEQUENCE LISTING (27 sequences)

SEQ ID NO: 1 - DNA, 6994 bp, Artificial Sequence
  pApl-pilA plasmid backbone including addA gene with homology arms and restriction sites for Asd (GGCGCGCC) and EcoRI (GAATTC)
gaattcacatacgcggccgcctgggccttgagctcgaatttcctgcattaatgaatcggccaacgcgcggggagaggcggtttgcgtattgggcgctcttccgcttcctcgctcactgactcgctgcgctcggtcgttcggctgcggcgagcggtatcagctcactcaaaggcggtaatacggttatccacagaatcaggggataacgcaggaaagaacatgtgagcaaaaggccagcaaaaggccaggaaccgtaaaaaggccgcgttgctggcgtttttccataggctccgcccccctgacgagcatcacaaaaatcgacgctcaagtcagaggtggcgaaacccgacaggactataaagataccaggcgtttccccctggaagctccctcgtgcgctctcctgttccgaccctgccgcttaccggatacctgtccgcctttctcccttcgggaagcgtggcgctttctcatagctcacgctgtaggtatctcagttcggtgtaggtcgttcgctccaagctgggctgtgtgcacgaaccccccgttcagcccgaccgctgcgccttatccggtaactatcgtcttgagtccaacccggtaagacacgacttatcgccactggcagcagccactggtaacaggattagcagagcgaggtatgtaggcggtgctacagagttcttgaagtggtggcctaactacggctacactagaagaacagtatttggtatctgcgctctgctgaagccagttaccttcggaaaaagagttggtagctcttgatccggcaaacaaaccaccgctggtagcggtggtttttttgtttgcaagcagcagattacgcgcagaaaaaaaggatctcaagaagatcctttgatcttttctacggggtctgacgctcagtggaacgaaaactcacgttaagggattttggtcatgagattatcaaaaaggatcttcacctagatccttttaaattaaaaatgaagttttaaatcaatctaaagtatatatgagtaaacttggtctgacagttaccaatgcttaatcagtgaggcacctatctcagcgatctgtctatttcgttcatccatagttgcctgactccccgtcgtgtagataactacgatacgggagggcttaccatctggccccagtgctgcaatgataccgcgagacccacgctcaccggctccagatttatcagcaataaaccagccagccggaagggccgagcgcagaagtggtcctgcaactttatccgcctccatccagtctattaattgttgccgggaagctagagtaagtagttcgccagttaatagtttgcgcaacgttgttgccattgctacaggcatcgtggtgtcacgctcgtcgtttggtatggcttcattcagctccggttcccaacgatcaaggcgagttacatgatcccccatgttgtgcaaaaaagcggttagctccttcggtcctccgatcgttgtcagaagtaagttggccgcagtgttatcactcatggttatggcagcactgcataattctcttactgtcatgccatccgtaagatgcttttctgtgactggtgagtactcaaccaagtcattctgagaatagtgtatgcggcgaccgagttgctcttgcccggcgtcaatacgggataataccgcgccacatagcagaactttaaaagtgctcatcattggaaaacgttcttcggggcgaaaactctcaaggatcttaccgctgttgagatccagttcgatgtaacccactcgtgcacccaactgatcttcagcatcttttactttcaccagcgtttctgggtgagcaaaaacaggaaggcaaaatgccgcaaaaaagggaataagggcgacacggaaatgttgaatactcatactcttcctttttcaatattattgaagcatttatcagggttattgtctcatgagcggatacatatttgaatgtatttagaaaaataaacaaataggggttccgcgcacatttccccgaaaagtgccacctgacgtctaagaaaccattattatcatgacattaacctataaaaataggcgtatcacgaggccctttcgtctcgcgcgtttcggtgatgacggtgaaaacctctgacacatgcagctcccggagacggtcacagcttgtctgtaagcggatgccaagcttgcatgcctgcaggtggcgcgccgaatgacgctaacagcaggacctatattgggaattaggttgaggagtccggcgagaatggcattggcgaaaattaaggggactctcagtatccacaagccgactactgttagtagggtgacaccaatcatgttgagtaaggcaccgattagccaacgacctagggctatttcgcaagtatcgagaatgtcgttcattcgccttcggtaaaaggcgggaattagttgtaagctgctgcgacggtaggcttgggggtcggctaaaagcatgagggtgaggacgaggattaataagatgctgactaatccttctactgtggttccgacgacgaccccaaaaccgccgattaattgattgctgagggcttgggcttgttggataatttgttcgatgcggatctgtctcaggtcgcgactgacttctgatagatattcccgtaagggtccgttgaggtcggtgcgtaaatagtcaattaacaggttcagcagctttagaccttgttcgagaccggcggggacctgtttggctagttgttctaattggttgattaggggggggactaccaataaaaagccgatggtaatccctaagaagaatagactaatggataggaagacggcaagcgatcgcggtagtttcagacgctggaattgacgggtgagacggtttaaggcggtggctaggacgacggcggcgaaaatcatcagcagggcttgtttaatccgccacaggatgtatatagcgattaagaaagctgtgaagcctatccatgtacctagggtcattgcgactgttgagggtgagagaatttgcttttctacaggcgatcgcctgtacaatagttatctatcatagaatactagattctgtggtgggattccaccaaagccagccagctacctatgacgcaacccagatatgatgaacaggaaaatatatctcgccacgcagcggtagatgaaggatgctgcgaggatatggaacgaaaatatgggtggaatcttgtgcgaattgaggtaacctcagatcctatccttgaggttgattgcgtatttctggggaaaacggagtttcctcggccctataatgaaactgataaggaggaagattgatgcgaaaatacatcatttttcgggctgataagggtgaacctggttggaaagaacgtaaactccaacatacccagggtttaactagaattttggctgaacatttcgactcttctgatcaacctattcctgagttgggatatcgaccgagggagtttattcgtattgatgggttgcataatcccactgaacatggctacagcacccattatcgtcagggtgactgggaagtaactagggtagaaagttactctcctgatgtgtctatggctgagtttgatatgatcgtgatttgcttttgcaaatatagccctgttaatggtcctgtgcaacctatgccagagcgtcgagtgtctgtagatgggttcgctggggatgagaagcggttggagcaatggcacgagtcccaaaagaaaccgactgaggtttagttggtccccggtttgcttatttgactagccagattcgccacgacaacagaaccgccagcagggaagaggggaatagaaccgcgaaaagagcgatcgcattggtttcgggaatggcgaaatttggcccgccatatttgatcagtaaggatagccctagggataggatcaggattttggccaccaataacagtttgttgtccatttatatataggatgcgatgggatgcgatcgcctatattttaccaattggtggcggccttaaccccctaagccctatgtctgacacccagtcaccccaaccgccttagtcggtattccccactgggtgggcgatacacgatttcccggaaaaattgaaaaaaaattttgtggcaggtgatatgatttgcgatcgaggtgggtaagttagaactacagaaaacaaataacctcatttcaccccgaggagaacgaattatgagggaagcggtgatcgccgaagtatcgactcaactatcagaggtagttggcgtcatcgagcgccatctcgaaccgacgttgctggccgtacatttgtacggctccgcagtggatggcggcctgaagccacacagtgatattgatttgctggttacggtgaccgtaaggcttgatgaaacaacgcggcgagctttgatcaacgaccttttggaaacttcggcttcccctggagagagcgagattctccgcgctgtagaagtcaccattgttgtgcacgacgacatcattccgtggcgttatccagctaagcgcgaactgcaatttggagaatggcagcgcaatgacattcttgcaggtatcttcgagccagccacgatcgacattgatctggctatcttgctgacaaaagcaagagaacatagcgttgccttggtaggtccagcggcggaggaactctttgatccggttcctgaacaggatctatttgaggcgctaaatgaaaccttaacgctatggaactcgccgcccgactgggctggcgatgagcgaaatgtagtgcttacgttgtcccgcatttggtacagcgcagtaaccggcaaaatcgcgccgaaggatgtcgctgccgactgggcaatggagcgcctgccggcccagtatcagcccgtcatacttgaagctagacaggcttatcttggacaagaagaagatcgcttggcctcgcgcgcagatcagttggaagaatttgtccactacgtgaaaggcgagatcaccaaggtagtcggcaaataacagataatctagcagtttaggtttcagatggagtcagctagggtctttaaccccatcgtcaactataagatggagagatggcatacggtgacactgttaaagccataactatattgctcttgttgataaaatcagaaactgaggccacttgagagtattgtaaataggtagtacagtagtgctacctattttgttttaaaataactaattgagtttatcgctgggactatggttgataatcagatgtcggaaaagcagaatattttatcagcagaagctgatatttacttgcataaaagggattatcaacaagcagccattttatatgaacaagccatcaatctcaatcccgactataaatataattactggaaactggggttaaccctgctgctacaggagcgggaggaagaagcccagaccacctggctggtggcgatgagtgatggagacccagaacagattgaccagtggacgatagacttactcgaggtgctatcatcagaagccgatgcacgaacctccgccgaagactattccgtggcttgggggattcgccaacacattttagaaataaacccccatggtattgataatatattaaagttaattgatttgtcaattaccctgacaacctataccggaaatgagatcgcagaatatggactggttcccttactgcaacaggagtccatcaatgtcaatccagatttactactgcacctgtggaaaaaactcctagttgtagatgcaattaatcccctatctctggaattgggagaggcggtgattaaccatcttggtgagcaaccggagtttgtcactagcttaatccctaaattatacgatattgcctattcctttggtgaaataggtatagccaagggctatggagagttgttgttgaacctggcaccgcatcatcaagagttgctgagggctctggctcaattttgtattcaattaaccgagtatgaccatggcattgaatatgccagacgttcctatcatctcactgaatccccagatcagcaagccctggatagcaattttatgatcagtggtctgatgtctcaagggggatgcacaaagcaagtgcgagaggtggtcaaccatcaggaatcattgctggatgctatgctgaaagacccgcccctagacttgggaactggggttatgcaattatataataccagctttttctttccttatgttagagattcacctgctgtcaactcacaaataaaagcccaagttgctcaaatttgccaagccaacttagaaacggctcaggcagaaaatatcgccacatatcaagcccggaatttacagaaacgccatcaatccgcgaccaatcaacccctaaaaattggttatatatcttattgtttccggcggcattctgtgggttggatatctcgctggttatttcaacatcacgatcgcgataaatttgaaatttatgcctatatgattggggcagaaaatcgacaagatgctctccaaaactggtatgcagaacaagccaacaagtcttatcaatatggaatagtaagcacagaagttgccgagcaaatttctgaagaccagattgatattctcattgatttagatagcctgacattaaccaatacctgcgccattatggcacttaaacccgcacctgtacaagtcacctggttgggatgggatgcctctgctatacccaccgttgactattttattgctgacccctatgttttgccagaaaatgcccaggattattactcagaaaccatctggcgactacctcaaacctatgtggccgtcggtggcttcgaggtcggcattcccagtttgcgaagagaggatatcaatattcccgaaaatgccattgtttattttaccgcccaaagggggccgaaatacaacccagaactagcccaattgcaaatgcaaattctgaaacaagtacccaatagttatttggtaattaagggattcgataaagagcaatc

SEQ ID NO: 2 - DNA, 5967 bp, Artificial Sequence
  pApl-pilA8005/aadA plasmid including aadA gene flanked by homology arms
gcctgggccttgagctcgaatttcctgcattaatgaatcggccaacgcgcggggagaggcggtttgcgtattgggcgctcttccgcttcctcgctcactgactcgctgcgctcggtcgttcggctgcggcgagcggtatcagctcactcaaaggcggtaatacggttatccacagaatcaggggataacgcaggaaagaacatgtgagcaaaaggccagcaaaaggccaggaaccgtaaaaaggccgcgttgctggcgtttttccataggctccgcccccctgacgagcatcacaaaaatcgacgctcaagtcagaggtggcgaaacccgacaggactataaagataccaggcgtttccccctggaagctccctcgtgcgctctcctgttccgaccctgccgcttaccggatacctgtccgcctttctcccttcgggaagcgtggcgctttctcatagctcacgctgtaggtatctcagttcggtgtaggtcgttcgctccaagctgggctgtgtgcacgaaccccccgttcagcccgaccgctgcgccttatccggtaactatcgtcttgagtccaacccggtaagacacgacttatcgccactggcagcagccactggtaacaggattagcagagcgaggtatgtaggcggtgctacagagttcttgaagtggtggcctaactacggctacactagaagaacagtatttggtatctgcgctctgctgaagccagttaccttcggaaaaagagttggtagctcttgatccggcaaacaaaccaccgctggtagcggtggtttttttgtttgcaagcagcagattacgcgcagaaaaaaaggatctcaagaagatcctttgatcttttctacggggtctgacgctcagtggaacgaaaactcacgttaagggattttggtcatgagattatcaaaaaggatcttcacctagatccttttaaattaaaaatgaagttttaaatcaatctaaagtatatatgagtaaacttggtctgacagttaccaatgcttaatcagtgaggcacctatctcagcgatctgtctatttcgttcatccatagttgcctgactccccgtcgtgtagataactacgatacgggagggcttaccatctggccccagtgctgcaatgataccgcgagacccacgctcaccggctccagatttatcagcaataaaccagccagccggaagggccgagcgcagaagtggtcctgcaactttatccgcctccatccagtctattaattgttgccgggaagctagagtaagtagttcgccagttaatagtttgcgcaacgttgttgccattgctacaggcatcgtggtgtcacgctcgtcgtttggtatggcttcattcagctccggttcccaacgatcaaggcgagttacatgatcccccatgttgtgcaaaaaagcggttagctccttcggtcctccgatcgttgtcagaagtaagttggccgcagtgttatcactcatggttatggcagcactgcataattctcttactgtcatgccatccgtaagatgcttttctgtgactggtgagtactcaaccaagtcattctgagaatagtgtatgcggcgaccgagttgctcttgcccggcgtcaatacgggataataccgcgccacatagcagaactttaaaagtgctcatcattggaaaacgttcttcggggcgaaaactctcaaggatcttaccgctgttgagatccagttcgatgtaacccactcgtgcacccaactgatcttcagcatcttttactttcaccagcgtttctgggtgagcaaaaacaggaaggcaaaatgccgcaaaaaagggaataagggcgacacggaaatgttgaatactcatactcttcctttttcaatattattgaagcatttatcagggttattgtctcatgagcggatacatatttgaatgtatttagaaaaataaacaaataggggttccgcgcacatttccccgaaaagtgccacctgacgtctaagaaaccattattatcatgacattaacctataaaaataggcgtatcacgaggccctttcgtctcgcgcgtttcggtgatgacggtgaaaacctctgacacatgcagctcccggagacggtcacagcttgtctgtaagcggatgccaagcttgcatgcctgcaggtggcgcgaacagaagacgaccaacactttctccctgatgggttgcgccctgatcaatgtcctttaaaccctgatacgttcttcaaccgtcgaacctagtccaaccgagtagcccataactgaccaccctatttaatcatgttgcattctgagcggaaccatgttcaaccccaaactatcccccaagttctcccggtccagtgaatctggctacaccctgcttgagtccatcatggctatggtggtggtcagcatcctgatggtcggcatttctccggtgttgggttttgccttcgccacacgggtacaggctcggcgcatagaactagccagcagagccgctaacagttatatcagtgctgtccgtactgacccaaccaataccaacttggtgctgttcaatcccagtgaccggaacgctggaccaactgcaactggtagcttgaactgtggggctggtcgagcctgtaccaccccagccaacttgttctgtgtggataatgacggaagtgggggatgtgaaaccgatagccccacggatatgattgttcagggaattggcataaatgagtgtagcgacgagctagagaatggttatcagttgattgtcagggtgtatcgtgctgacgcatttgcccaatcgggacaactagagggggctaatgatgacgggtctagtaatttagcgagttcccgagtcggtttaggaaaccccagagaccccctagtgcaggtgcgaaccgagattagccccactagcaccagttcctttgggagtttacgtgaccgtttagcaggatgcagttctgacgatgaaggggattaataggtttggtgatggttcccatggagtgcaaaagtaagattatcccggtagagaggtagttatgctgtccctagttcggttttggttaatttgtgtattgaaatctaggtcaaaaaccacccaggggaatgacttaggcttcacgatgattgagttattgatttcggctgttgtggctagtatgatcatcacgcccatcctattctttgtggtggatgttttacgaaccgatacccgggaagaaatcacagccagatcggaacaggagttacaggcggcagcagatttcattcgtcgcgacctctcccaggctatctatatctacgacggtgaaggggttaatgcgattaggagccaacttcctgattccgataatgtggtattggtgttctggaaacaggagtttcgcgaaggtgtgattcctcacggtgacgtccccaggccagttgctgctaatcattgcgatacgaggcgttgcgatgatgtccaagttttatctttagttgcttactatttacaaacagaaagagagcctaatagtccttggtctgatcaggcgcgtatttctcgcttacaaatcaacgatggtgtcatcgatccgaatccagaagatgaatgcacccaaccaccatgttatgtcaaactgggtgataaggaattcaaaccagaccgaggttttgatcgacctcctggccgtacaagcatgaatgcttgggaagcaaaagagggcgagcagattgaagcatcacgagaagttctgattgattacatagacaaaacagaactaacaggtgatatagattgtgaatctcgtggcatcagtaatgatgatagtgaggatttactatccgtgggtaagaattctgaggggaatcctatctatggcttttttgtatgtgtagactcccgtaatacagcagctttagttaacctgagaatgaatgcggcaattcgcattgatccgaatgctacagaattcgacgaggataggcgatcgctttttccagagaccagctttttggttaaaggcttaggtgttttcaattaaccgataaaatcagggaatttataataaaaggaacctataaaatgagtattttaattaacccaaaatcggtgaatcccaggcgcaccaaaaaccagtcgggcttcaccatcattgagacgttggtggtagttttaatgagggaagcggtgatcgccgaagtatcgactcaactatcagaggtagttggcgtcatcgagcgccatctcgaaccgacgttgctggccgtacatttgtacggctccgcagtggatggcggcctgaagccacacagtgatattgatttgctggttacggtgaccgtaaggcttgatgaaacaacgcggcgagctttgatcaacgaccttttggaaacttcggcttcccctggagagagcgagattctccgcgctgtagaagtcaccattgttgtgcacgacgacatcattccgtggcgttatccagctaagcgcgaactgcaatttggagaatggcagcgcaatgacattcttgcaggtatcttcgagccagccacgatcgacattgatctggctatcttgctgacaaaagcaagagaacatagcgttgccttggtaggtccagcggcggaggaactctttgatccggttcctgaacaggatctatttgaggcgctaaatgaaaccttaacgctatggaactcgccgcccgactgggctggcgatgagcgaaatgtagtgcttacgttgtcccgcatttggtacagcgcagtaaccggcaaaatcgcgccgaaggatgtcgctgccgactgggcaatggagcgcctgccggcccagtatcagcccgtcatacttgaagctagacaggcttatcttggacaagaagaagatcgcttggcctcgcgcgcagatcagttggaagaatttgtccactacgtgaaaggcgagatcaccaaggtagtcggcaaataagtagttataactagccaattgtaacacaaaaaattaattatctactgaatattttacaaaactttacccccaatttcggaaaacatagtttagaatacaccaccaaagatatcacccgtaacgaggccttttacgagtgagattagttgtgtatgctgcggttagctgacctacacgacatctatccttgtgacccaggttaaataatggaaaatacattaattaagcacttgcttctggttcagaaacaggctattaatttagtgcctgaaaaacctgttagcagtgactatcagggtgcgaaatcgcgaaaatcctctacagaatcagggttttctttgttagaagtgttaggggtgatggtgattatatcaatactaggtgggatagcggttccgacttggttaggtttcgcgaataaccagaaactgcaaacctctatccggcgactcaactgggctatccactcagccaaaagtgaggctatactatctagtacatcatggcaagcgagtatcagggaatatgggggacgagtacaggtagcagtccatcccgcgaagactccccctggtcaactcccagaaggttcatggactaacctagaaccggggatagaaattgacaaccgggaaaggaacaccaggaataaatatgaaactaccctgcgaagagtagacccggacaccaaccaagtccgaaacgcggggacggtgtaccgagttttattcaactaccaaggctgtccggtctataacccgtctaatttatgcacgcaaacttctctagctgcgaagggacgcattgctatccatcatcctgaagttccaggtcaaaagcgatgtatcatcatttcgacgctgataggtgcgactcgcattggtcagcaacagcaaagaccggatcaaaatggctactattgccattaattaataattaataattaataattaataattattaattgggtagcgaccctgtgggcc

SEQ ID NO: 3 - DNA, 8117 bp, Artificial Sequence
  pApl-NS1/Prs-crtW-crtZ plasmid including aadA gene, crtW, crtZ, and homology arms
gcctgggccttgagctcgaatttcctgcattaatgaatcggccaacgcgcggggagaggcggtttgcgtattgggcgctcttccgcttcctcgctcactgactcgctgcgctcggtcgttcggctgcggcgagcggtatcagctcactcaaaggcggtaatacggttatccacagaatcaggggataacgcaggaaagaacatgtgagcaaaaggccagcaaaaggccaggaaccgtaaaaaggccgcgttgctggcgtttttccataggctccgcccccctgacgagcatcacaaaaatcgacgctcaagtcagaggtggcgaaacccgacaggactataaagataccaggcgtttccccctggaagctccctcgtgcgctctcctgttccgaccctgccgcttaccggatacctgtccgcctttctcccttcgggaagcgtggcgctttctcatagctcacgctgtaggtatctcagttcggtgtaggtcgttcgctccaagctgggctgtgtgcacgaaccccccgttcagcccgaccgctgcgccttatccggtaactatcgtcttgagtccaacccggtaagacacgacttatcgccactggcagcagccactggtaacaggattagcagagcgaggtatgtaggcggtgctacagagttcttgaagtggtggcctaactacggctacactagaagaacagtatttggtatctgcgctctgctgaagccagttaccttcggaaaaagagttggtagctcttgatccggcaaacaaaccaccgctggtagcggtggtttttttgtttgcaagcagcagattacgcgcagaaaaaaaggatctcaagaagatcctttgatcttttctacggggtctgacgctcagtggaacgaaaactcacgttaagggattttggtcatgagattatcaaaaaggatcttcacctagatccttttaaattaaaaatgaagttttaaatcaatctaaagtatatatgagtaaacttggtctgacagttaccaatgcttaatcagtgaggcacctatctcagcgatctgtctatttcgttcatccatagttgcctgactccccgtcgtgtagataactacgatacgggagggcttaccatctggccccagtgctgcaatgataccgcgagacccacgctcaccggctccagatttatcagcaataaaccagccagccggaagggccgagcgcagaagtggtcctgcaactttatccgcctccatccagtctattaattgttgccgggaagctagagtaagtagttcgccagttaatagtttgcgcaacgttgttgccattgctacaggcatcgtggtgtcacgctcgtcgtttggtatggcttcattcagctccggttcccaacgatcaaggcgagttacatgatcccccatgttgtgcaaaaaagcggttagctccttcggtcctccgatcgttgtcagaagtaagttggccgcagtgttatcactcatggttatggcagcactgcataattctcttactgtcatgccatccgtaagatgcttttctgtgactggtgagtactcaaccaagtcattctgagaatagtgtatgcggcgaccgagttgctcttgcccggcgtcaatacgggataataccgcgccacatagcagaactttaaaagtgctcatcattggaaaacgttcttcggggcgaaaactctcaaggatcttaccgctgttgagatccagttcgatgtaacccactcgtgcacccaactgatcttcagcatcttttactttcaccagcgtttctgggtgagcaaaaacaggaaggcaaaatgccgcaaaaaagggaataagggcgacacggaaatgttgaatactcatactcttcctttttcaatattattgaagcatttatcagggttattgtctcatgagcggatacatatttgaatgtatttagaaaaataaacaaataggggttccgcgcacatttccccgaaaagtgccacctgacgtctaagaaaccattattatcatgacattaacctataaaaataggcgtatcacgaggccctttcgtctcgcgcgtttcggtgatgacggtgaaaacctctgacacatgcagctcccggagacggtcacagcttgtctgtaagcggatgccaagcttgcatgcctgcaggtggcgcgccaggtccgaagaagaacgcaccatagctgctggtaaagaagcccgcgccagggctgaacaactcctgcaaactgtccgcgctgagttggaaaggttgcgactcgaagctgataccgtcctacctgcagaggcggagcgagaagccagagaactgcaagccagaggtaatgcggccgctttagcggaaaattcccgcgcggcggcggaagtaaacgacctgattaacgcagtttggcaggaaatgggcgacgacgcatcggaactgttttacttacaacaaattgagatggtcttgcgcgaagctgcccaaattccccgccgggttagtctggaatatgtcaatgttattgatagtggagacggggaagcgatcgctggtttggttcgcgcctatcccgaaattttccgccaattcctcgaaagtgtcgatcgcactttgggtattaatgtatctaggactttgggggaacataacaagcagaaattaaataacaattagtcaatttgatggcaaccaaacacaggtacaggaattatggaaattatcatcgccttattagcagccctgggtttaggaaccggagcgactgtatttattatccgcaatctctactatatttgtcagcctagcgaagtgttgatttttgccggaggtcgtcgccctacacaagatgatcgcactgtgggatatcgcctggtgaaaggtggtagcagcattcggacacccctgctagaacaagcctttcacatggatttaaccaatatgattattgagttaaaggtggctaatgcttactcgaaaggaggcattcctttacaggttgatggggtggcgaatattaaaattgctggggaagaacccacaattcataatgcgatcgagcgtttgttggggaaaactcgccaggaaattgaacgcattgctaaagataccctggaaggaaacctgcgcggggtattagccagccttactcctgaacaggttaatggggataaattggcttttgctaaaagtctcctcgaagaagctgaggatgacttagaacaactggggctgattttagatactctccaaattcaaaatatttctgatgacgtgggatatcttgactccatcggacgacaacaacgggcggaattgtttagagattctcgtgtcgctgaagcacaagctaaggctgatgctgctatccgtactgcggaaaatcataaaatgactcagttgaaaaagttggaaactgaggtagaggtatctaaggcggaagctgaacgccgggtggctgatgctatgactaaacgggcggcggtggtagcagagtcggagtcggaaacagcggctgaggtggctaggactcaggctgaggtctctgttcaaaaagaaaggattaagcaggtagaacagcaactacaagctgatgtggtcgcaccagcagaggcggaatgtaaaaaggcgatcgctagggcgcggggggatgctgcccaaattattgaagatgggaaagcacaagctgaagggacacgacgactggctgagtcttggaaagcagccggtcggaccgtcactgcataattcgtgtcgctcaaggcgcactcccgttctggataatgttttttgcgccgacatcataacggttctggcaaatattctgaaatgagctgttgacaattaatcatccggctcgtataatgtgtggaattgtgagcggataacaatttcatacgctcacaattggtaccggtgataccagcatcgtcttgatgcccttggcagcaccctgctaaggaggcaacaagatgacggctgcggtcgctgagccgcgaatcgtgcctcgtcaaacctggatcgggctcacacttgcagggatgattgtggcaggctgggggagtcttcacgtctatggagtctactttcatcgctgggggacaagtagcctcgttattgtgccagcaatcgtggctgtccagacctggctcagtgtgggcctattcattgtcgcacacgacgctatgcacgggtcgctggcgccgggtcggcctcgcctaaacgcagccgtaggcagactcaccttagggctctatgccggtttccgatttgatcgccttaaaacggcccaccacgcacatcacgccgcccccggtactgccgatgaccctgatttctacgccccagcaccgcgagcgtttttgccttggttcctcaacttctttcgcacttactttggctggcgtgagatggctgttctgacagctttagtcctaatagccttgtttggtttgggtgcccggccggcaaatcttctcacgttctgggcagctccggcgctgttaagtgctctacagctattcacttttggcacgtggctgccgcaccgccacactgatcagccttttgcggacgcccaccatgctcggtcttccggttacggcccggtgctcagcctgcttacctgttttcactttggtcggcaccacgaacaccatctgacaccgtggcgcccctggtggcggctatggcgaggtgagagctaaacacaggaaacaggaattagatatgctgtggatttggaacgcgctgatcgtgtttgtcacagtcatcgggatggaagttattgccgccttggcacacaaatacatcatgcacggctggggctggggatggcatctgtctcaccacgaaccccgcaaaggcgctttcgaagtcaatgatctgtatgctgtcgtgtttgcagccctgagcattttgctcatctacctgggctcgaccggtatgtggccgttgcaatggattggtgccggcatgaccgcctacggtctgctgtatttcatggtgcacgatggcctggtccatcaacggtggccttttcggtatattccccgaaagggctacctgaagcgcctatatatggcccatcgaatgcatcacgcagtccgggggaaggaagggtgtgtgagttttgggtttctatatgctcccccgttgtcgaaactgcaagcaaccctgcgtgagcgtcatggcgctcgcgctggggcggcgcgggacgcgcaagggggcgaagatgaaccggcatcggggaaataaactagtcatcgagctagcaagcttggccggatccggccggatccggagtttgtagaaacgcaaaaaggccatccgtcaggatggccttctgcttaatttgatgcctggcagtttatggcgggcgtcctgcccgccaccctccgggccgttgcttcgcaacgttcaaatccgctcccggcggatttgtcctactcaggagagcgttcaccgacaaacaacagataaaacgaaaggcccagtctttcgactgagcctttcgttttatttgatgcctggcagttccctactctcgagtcaccccaaccgccttagtcggtattccccactgggtgggcgatacacgatttcccggaaaaattgaaaaaaaattttgtggcaggtgatatgatttgcgatcgaggtgggtaagttagaactacagaaaacaaataacctcatttcaccccgaggagaacgaattatgagggaagcggtgatcgccgaagtatcgactcaactatcagaggtagttggcgtcatcgagcgccatctcgaaccgacgttgctggccgtacatttgtacggctccgcagtggatggcggcctgaagccacacagtgatattgatttgctggttacggtgaccgtaaggcttgatgaaacaacgcggcgagctttgatcaacgaccttttggaaacttcggcttcccctggagagagcgagattctccgcgctgtagaagtcaccattgttgtgcacgacgacatcattccgtggcgttatccagctaagcgcgaactgcaatttggagaatggcagcgcaatgacattcttgcaggtatcttcgagccagccacgatcgacattgatctggctatcttgctgacaaaagcaagagaacatagcgttgccttggtaggtccagcggcggaggaactctttgatccggttcctgaacaggatctatttgaggcgctaaatgaaaccttaacgctatggaactcgccgcccgactgggctggcgatgagcgaaatgtagtgcttacgttgtcccgcatttggtacagcgcagtaaccggcaaaatcgcgccgaaggatgtcgctgccgactgggcaatggagcgcctgccggcccagtatcagcccgtcatacttgaagctagacaggcttatcttggacaagaagaagatcgcttggcctcgcgcgcagatcagttggaagaatttgtccactacgtgaaaggcgagatcaccaaggtagtcggcaaataactagctggcctggaagggtgggaaagtgttaacaactggttgacaatattccgcttttccaggtcttgtcgaagtacgactacgggtattgatgtggcgacggctgttcaaaattggggcggcggttcttctcaacctcaacctacttccacagctaaaagtctcaaatcttcccgcactaatggtcaagctgttcgccgcactaatggcgcagcacctaagccagaagatactacacaaagcctacagagcgaggttaaacaactacttgatcatgtcgcacaaaatactaagaataatgctgaggctgaagaggcgatcgcccaggctttgcgacagtatcctaacctcaagcgtcgtttacagatgctttttaagtctcagggaactcaggcgatccgaaatatgtttaatcaccctactatctacatccctaccgctatgctgcaaatgtggctagaacaggattagagcgtattcccccccctctcgtctagggtgggggatctgtctctgtaactgtatatgcacaaaatggcgtttttgtcaataagccgaaaaatggaccccgcttttaaccccaaaactcgtgcatcgccagttttattttttggtaagataataattataaccgcgacaaaataagggttttagcctttatttttggaaatagacacagtaagcccttgggtgcgatttccttgagcataccataacccccataatctcgtcaactttttgcgaggtatttgccataaaattgtattaattcttaacaatattttaaaaataaaatctatctagccgtataaattagtaaaatttatgtaatttcccgattgagggggtggggtgtgggggggtttatagtcaaattaatgtgattggatctcatttaacctctgacgtactacttgcatatcctgccacattaaccatttaggtttaccaacatctcgcgaggaatttctgagtaggtatgcagggtgaaaaatcggcatacattgacgaccttcccactgaaaccactgaccgcgaattttagtaatcgggcgtttatctcctagaatagacttaactgcagtcgccccagttaggaggataatttgaggattaatgaggcggatttgttctaatagataaggcttacaggcttggagttctgaagcggttggggtgcgattttccgggggacgacagcggatagcattagaaatataaacttcggtatctgtactcagtcctacggagtctaaaatattatcaagaagttttccagatctaccgacaaacggaagaccttgttcatcttcatgttgtcctggtgcttctccgataatcataatgggggcggtggggttccctcgaccaatcacagcatgagtgcggttttttccaagttcacagcgcgagcacctattacaatgatcggcaatttgtgcgagagtttgataggttcccggcggtatgggagtcttggcattttggggaatttcttctaggtcaaaatctaccgacttaggggattgtaatgggtcttgattaacactaagaatatcgaacaggctgagttgttgggaattcacatacgcggcc

SEQ ID NO: 4 - DNA, 8146 bp, Artificial Sequence
  pApl-NS1/aadA-cpcBA plasmid backbone including aadA, cpcA, and cpcB genes with a p15A origin of replication
aggtccgaagaagaacgcaccatagctgctggtaaagaagcccgcgccagggctgaacaactcctgcaaactgtccgcgctgagttggaaaggttgcgactcgaagctgataccgtcctacctgcagaggcggagcgagaagccagagaactgcaagccagaggtaatgcggccgctttagcggaaaattcccgcgcggcggcggaagtaaacgacctgattaacgcagtttggcaggaaatgggcgacgacgcatcggaactgttttacttacaacaaattgagatggtcttgcgcgaagctgcccaaattccccgccgggttagtctggaatatgtcaatgttattgatagtggagacggggaagcgatcgctggtttggttcgcgcctatcccgaaattttccgccaattcctcgaaagtgtcgatcgcactttgggtattaatgtatctaggactttgggggaacataacaagcagaaattaaataacaattagtcaatttgatggcaaccaaacacaggtacaggaattatggaaattatcatcgccttattagcagccctgggtttaggaaccggagcgactgtatttattatccgcaatctctactatatttgtcagcctagcgaagtgttgatttttgccggaggtcgtcgccctacacaagatgatcgcactgtgggatatcgcctggtgaaaggtggtagcagcattcggacacccctgctagaacaagcctttcacatggatttaaccaatatgattattgagttaaaggtggctaatgcttactcgaaaggaggcattcctttacaggttgatggggtggcgaatattaaaattgctggggaagaacccacaattcataatgcgatcgagcgtttgttggggaaaactcgccaggaaattgaacgcattgctaaagataccctggaaggaaacctgcgcggggtattagccagccttactcctgaacaggttaatggggataaattggcttttgctaaaagtctcctcgaagaagctgaggatgacttagaacaactggggctgattttagatactctccaaattcaaaatatttctgatgacgtgggatatcttgactccatcggacgacaacaacgggcggaattgtttagagattctcgtgtcgctgaagcacaagctaaggctgatgctgctatccgtactgcggaaaatcataaaatgactcagttgaaaaagttggaaactgaggtagaggtatctaaggcggaagctgaacgccgggtggctgatgctatgactaaacgggcggcggtggtagcagagtcggagtcggaaacagcggctgaggtggctaggactcaggctgaggtctctgttcaaaaagaaaggattaagcaggtagaacagcaactacaagctgatgtggtcgcaccagcagaggcggaatgtaaaaaggcgatcgctagggcgcggggggatgctgcccaaattattgaagatgggaaagcacaagctgaagggacacgacgactggctgagtcttggaaagcagccggtagtcaccccaaccgccttagtcggtattccccactgggtgggcgatacacgatttcccggaaaaattgaaaaaaaattttgtggcaggtgatatgatttgcgatcgaggtgggtaagttagaactacagaaaacaaataacctcatttcaccccgaggagaacgaattatgagggaagcggtgatcgccgaagtatcgactcaactatcagaggtagttggcgtcatcgagcgccatctcgaaccgacgttgctggccgtacatttgtacggctccgcagtggatggcggcctgaagccacacagtgatattgatttgctggttacggtgaccgtaaggcttgatgaaacaacgcggcgagctttgatcaacgaccttttggaaacttcggcttcccctggagagagcgagattctccgcgctgtagaagtcaccattgttgtgcacgacgacatcattccgtggcgttatccagctaagcgcgaactgcaatttggagaatggcagcgcaatgacattcttgcaggtatcttcgagccagccacgatcgacattgatctggctatcttgctgacaaaagcaagagaacatagcgttgccttggtaggtccagcggcggaggaactctttgatccggttcctgaacaggatctatttgaggcgctaaatgaaaccttaacgctatggaactcgccgcccgactgggctggcgatgagcgaaatgtagtgcttacgttgtcccgcatttggtacagcgcagtaaccggcaaaatcgcgccgaaggatgtcgctgccgactgggcaatggagcgcctgccggcccagtatcagcccgtcatacttgaagctagacaggcttatcttggacaagaagaagatcgcttggcctcgcgcgcagatcagttggaagaatttgtccactacgtgaaaggcgagatcaccaaggtagtcggcaaataactagctggcctggaagggtgggaaagtgttaacaactggttgacaatattccgcttttccaggtcttgtcgaagtacgcggaccgttgaaggggtgagaaggaaggcgaatgttgatttatgaagtttgattaacatttgtatcaaaatataaaattcttctcataaaccctgtacaatcttttaagatttcggaaagtgttctaggatactgaagaaatgaaccacggggcaattgttaaaagcctttgtcgatggttcgccccggaaggggtcttaggaggtgacaccgatggattgattgtcgtgatcattcatggtgtgtccaatcccaactcaactctaagcaagtcaacaagtaggagataaatccatgtttgatgccttcaccaaggtggtttctcaagctgatactcgcggcgaaatgctgagtacagctcaaatcgatgctctgagccaaatggttgctgaaagcaacaaacgtttggattctgttaaccgcattaccagcaacgcttccaccattgtttccaacgctgctcgttctttgttcgcagagcaaccccaactgattgctcccggtggaaacgcctacaccagccgtcgtatggctgcttgcttgcgtgacatggaaatcatcctgcgctatgtaacctacgctgtgtttgctggcgatgcaagtgttctcgaagatcgttgcttgaacggtttgcgtgaaacttacctggctttgggaactcccggttcttccgttgctgtcggtgttggcaaaatgaaagaagctgctctggcgatcgttaacgatcccgcaggtatcactcctggtgattgtagcgctttggcttcagaaatcgctggttactttgaccgtgctgctgcagcagtttcctaatcaagcagatccatagcatataacaattgaaacagtttagctgaagtctaagtgactggacttctgtttgttacctaattttttgtaaaccaatcgggagataactcgagaatgaaaacccccctaaccgaagcagtttctatcgctgattcccaaggtcgtttcctaagcagcaccgaaatccaagtagcttttggccgttttcgtcaagccaaagctggtctggaagctgctaaagctttgacctctaaagctgatagtctgatcagtggtgctgcccaagcagtgtacaacaagttcccctacaccacccaaatgcagggacctaactacgcggcagaccaacgcggtaaggacaaatgtgctcgtgacataggctactacctgcggatggtaacttattgcctgattgctggtggaactggccccatggatgagtacctgattgccggtattgatgaaatcaaccggactttcgagctttctccaagctggtacattgaagccctgaaatacatcaaagctaaccacggtttgtctggtgacgctgctgttgaagctaactcctacctcgactacgcgatcaacgccctgagctagactagtcatcgagctagcaagcttggccggatccggccggatccggagtttgtagaaacgcaaaaaggccatccgtcaggatggccttctgcttaatttgatgcctggcagtttatggcgggcgtcctgcccgccaccctccgggccgttgcttcgcaacgttcaaatccgctcccggcggatttgtcctactcaggagagcgttcaccgacaaacaacagataaaacgaaaggcccagtctttcgactgagcctttcgttttatttgatgcctggcagttccctactctcgactacgggtattgatgtggcgacggctgttcaaaattggggcggcggttcttctcaacctcaacctacttccacagctaaaagtctcaaatcttcccgcactaatggtcaagctgttcgccgcactaatggcgcagcacctaagccagaagatactacacaaagcctacagagcgaggttaaacaactacttgatcatgtcgcacaaaatactaagaataatgctgaggctgaagaggcgatcgcccaggctttgcgacagtatcctaacctcaagcgtcgtttacagatgctttttaagtctcagggaactcaggcgatccgaaatatgtttaatcaccctactatctacatccctaccgctatgctgcaaatgtggctagaacaggattagagcgtattcccccccctctcgtctagggtgggggatctgtctctgtaactgtatatgcacaaaatggcgtttttgtcaataagccgaaaaatggaccccgcttttaaccccaaaactcgtgcatcgccagttttattttttggtaagataataattataaccgcgacaaaataagggttttagcctttatttttggaaatagacacagtaagcccttgggtgcgatttccttgagcataccataacccccataatctcgtcaactttttgcgaggtatttgccataaaattgtattaattcttaacaatattttaaaaataaaatctatctagccgtataaattagtaaaatttatgtaatttcccgattgagggggtggggtgtgggggggtttatagtcaaattaatgtgattggatctcatttaacctctgacgtactacttgcatatcctgccacattaaccatttaggtttaccaacatctcgcgaggaatttctgagtaggtatgcagggtgaaaaatcggcatacattgacgaccttcccactgaaaccactgaccgcgaattttagtaatcgggcgtttatctcctagaatagacttaactgcagtcgccccagttaggaggataatttgaggattaatgaggcggatttgttctaatagataaggcttacaggcttggagttctgaagcggttggggtgcgattttccgggggacgacagcggatagcattagaaatataaacttcggtatctgtactcagtcctacggagtctaaaatattatcaagaagttttccagatctaccgacaaacggaagaccttgttcatcttcatgttgtcctggtgcttctccgataatcataatgggggcggtggggttccctcgaccaatcacagcatgagtgcggttttttccaagttcacagcgcgagcacctattacaatgatcggcaatttgtgcgagagtttgataggttcccggcggtatgggagtcttggcattttggggaatttcttctaggtcaaaatctaccgacttaggggattgtaatgggtcttgattaacactaagaatatcgaacaggctgagttgttgggaattcacatacgcggccgcctgggccttgagctcgaatttcctgcattaatgaatcggccaacgcgcggggagaggcggtttgcgtattgggcgctcttccgcttcctcgctcactgactcgctgcgctcggtcgttcggctgcggcgagcggtatcagctcactcaaaggcggtaatacggttatccacagaatcaggggataacgcaggaaagaacatgtgagcaaaaggccagcaaaaggccaggaaccgtaaaaatagcggagtgtatactggcttactatgttggcactgatgagggtgtcagtgaagtgcttcatgtggcaggagaaaaaaggctgcaccggtgcgtcagcagaatatgtgatacaggatatattccgcttcctcgctcactgactcgctacgctcggtcgttcgactgcggcgagcggaaatggcttacgaacggggcggagatttcctggaagatgccaggaagatacttaacagggaagtgagagggccgcggcaaagccgtttttccataggctccgcccccctgacaagcatcacgaaatctgacgctcaaatcagtggtggcgaaacccgacaggactataaagataccaggcgtttccccctggcggctccctcgtgcgctctcctgttcctgcctttcggtttaccggtgtcattccgctgttatggccgcgtttgtctcattccacgcctgacactcagttccgggtaggcagttcgctccaagctggactgtatgcacgaaccccccattcagtccgaccgctgcgccttatccggtaactatcgtcttgagtccaacccggaaagacatgcaaaagcaccactggcagcagccactggtaattgatttagaggagttagtcttgaagtcatgcgccggttaaggctaaactgaaaggacaagttttggtgactgcgctcctccaagccagttacctcggttcaaagagttggtagctcagagaaccttcgaaaaaccgccctgcaaggcggttttttcgttttcagagcaagagattacgcgcagaccaaaacgatctcaagaagatcatcttattaagattatcaaaaaggatcttcacctagatccttttaaattaaaaatgaagttttaaatcaatctaaagtatatatgagtaaacttggtctgacagttaccaatgcttaatcagtgaggcacctatctcagcgatctgtctatttcgttcatccatagttgcctgactccccgtcgtgtagataactacgatacgggagggcttaccatctggccccagtgctgcaatgataccgcgagacccacgctcaccggctccagatttatcagcaataaaccagccagccggaagggccgagcgcagaagtggtcctgcaactttatccgcctccatccagtctattaattgttgccgggaagctagagtaagtagttcgccagttaatagtttgcgcaacgttgttgccattgctacaggcatcgtggtgtcacgctcgtcgtttggtatggcttcattcagctccggttcccaacgatcaaggcgagttacatgatcccccatgttgtgcaaaaaagcggttagctccttcggtcctccgatcgttgtcagaagtaagttggccgcagtgttatcactcatggttatggcagcactgcataattctcttactgtcatgccatccgtaagatgcttttctgtgactggtgagtactcaaccaagtcattctgagaatagtgtatgcggcgaccgagttgctcttgcccggcgtcaatacgggataataccgcgccacatagcagaactttaaaagtgctcatcattggaaaacgttcttcggggcgaaaactctcaaggatcttaccgctgttgagatccagttcgatgtaacccactcgtgcacccaactgatcttcagcatcttttactttcaccagcgtttctgggtgagcaaaaacaggaaggcaaaatgccgcaaaaaagggaataagggcgacacggaaatgttgaatactcatactcttcctttttcaatattattgaagcatttatcagggttattgtctcatgagcggatacatatttgaatgtatttagaaaaataaacaaataggggttccgcgcacatttccccgaaaagtgccacctgacgtctaagaaaccattattatcatgacattaacctataaaaataggcgtatcacgaggccctttcgtctcgcgcgtttcggtgatgacggtgaaaacctctgacacatgcagctcccggagacggtcacagcttgtctgtaagcggatgccaagcttgcatgcctgcaggtggcgcgcc

SEQ ID NO: 5 - protein, 458 aa, Acinetobacter baylii sp.
MRPLHPIDFIFLSLEKRQQPMHVGGLFLFQIPDNAPDTFIQDLVNDIRISKSIPVPPFNNKLNGLFWDEDEEFDLDHHFRHIALPHPGRIRELLIYISQEHSTLLDRAKPLWTCNIIEGIEGNRFAMYFKIHHAMVDGVAGMRLIEKSLSHDVTEKSIVPPWCVEGKRAKRLREPKTGKIKKIMSGIKSQLQATPTVIQELSQTVFKDIGRNPDHVSSFQAPCSILNQRVSSSRRFAAQSFDLDRFRNIAKSLNVTINDVVLAVCSGALRAYLMSHNSLPSKPLIAMVPASIRNDDSDVSNRITMILANLATHKDDPLQRLEIIRRSVQNSKQRFKRMTSDQILNYSAVVYGPAGLNIISGMMPKRQAFNLVISNVPGPREPLYWNGAKLDALYPASIVLDGQALNITMTSYLDKLEVGLIACRNALPRMQNLLTHLEEEIQLFEGVIAKQEDIKTAN

SEQ ID NO: 6 - protein, 446 aa, Streptomyces coelicolor
MTPDPLAPLDLAFWNIESAEHPMHLGALGVFEADSPTAGALAADLLAARAPAVPGLRMRIRDTWQPPMALRRPFAFGGATREPDPRFDPLDHVRLHAPATDFHARAGRLMERPLERGRPPWEAHVLPGADGGSFAVLFKFHHALADGLRALTLAAGVLDPMDLPAPRPRPEQPPRGLLPDVRALPDRLRGALSDAGRALDIGAAAALSTLDVRSSPALTAASSGTRRTAGVSVDLDDVHHVRKTTGGTVNDVLIAVVAGALRRWLDERGDGSEGVAPRALIPVSRRRPRSAHPQGNRLSGYLMRLPVGDPDPLARLGTVRAAMDRNKDAGPGRGAGAVALLADHVPALGHRLGGPLVSGAARLWFDLLVTSVPLPSLGLRLGGHPLTEVYPLAPLARGHSLAVAVSTYRGRVHYGLLADAKAVPDLDRLAVAVAEEVETLLTACRP

SEQ ID NO: 7 - protein, 457 aa, Alcanivorax borkumensis
MKALSPVDQLFLWLEKRQQPMHVGGLQLFSFPEGAGPKYVSELAQQMRDYCHPVAPFNQRLTRRLGQYYWTRDKQFDIDHHFRHEALPKPGRIRELLSLVSAEHSNLLDRERPMWEAHLIEGIRGRQFALYYKIHHSVMDGISAMRIASKTLSTDPSEREMAPAWAFNTKKRSRSLPSNPVDMASSMARLTASISKQAATVPGLAREVYKVTQKAKKDENYVSIFQAPDTILNNTITGSRRFAAQSFPLPRLKVIAKAYNCTINTVVLSMCGHALREYLISQHALPDEPLIAMVPMSLRQDDSTGGNQIGMILANLGTHICDPANRLRVIHDSVEEAKSRFSQMSPEEILNFTALTMAPTGLNLLTGLAPKWRAFNVVISNIPGPKEPLYWNGAQLQGVYPVSIALDRIALNITLTSYVDQMEFGLIACRRTLPSMQRLLDYLEQSIRELEIGAGIK

SEQ ID NO: 8 - DNA, 2595 bp, Artificial Sequence
  Codon-optimized S. cerevisiae phosphatidate phosphatase (PAH1)
atggaattccaatatgttggtcgggctttgggtagtgttagtaaaacgtggtcgagtatcaaccccgccaccctgagcggcgctatcgatgtcattgtcgtggaacaccccgatggccggctcagttgtagccccttccatgtgcgctttggtaaattccagattctgaaacccagccaaaagaaagtccaggtctttattaacgagaaactgtcgaatatgcccatgaaactctcggatagcggcgaggcgtacttcgtttttgagatgggtgatcaagtgacggatgtcccggatgaactgctcgtctcgccggtcatgagtgccacgagtagtccgccccaatcgccggaaacctcgattctcgaaggcggtaccgaaggcgagggcgaaggtgagaatgaaaataagaaaaaggaaaagaaggtgttggaggagcccgactttctggacattaatgacaccggtgacagcggcagcaagaacagtgagacgacgggttcgctctcgccgaccgaaagtagtacgacgacgccgcccgatagcgtcgaggaacgcaagttggtcgaacaacggaccaagaattttcagcaaaagctgaataagaaactgaccgaaatccatattccgagcaaattggacaataacggtgatttgctcctggacaccgagggttataagccgaataaaaacatgatgcacgacacggatattcagctgaagcaattgctcaaggatgagttcggtaacgatagcgatatttcgagcttcatcaaagaagacaagaatggcaacattaaaatcgtgaacccctatgagcatttgaccgatttgagtcccccgggtacgcccccgaccatggccacgagtggcagtgtcctgggcttggatgcgatggagagtggttcgacgctgaacagcttgagcagcagcccgagcggcagtgacaccgaggatgagacgagctttagcaaggaacagtcgtcgaagagtgaaaaaacgtcgaagaaaggcaccgcgggttcgggtgaaacggagaaacgctacatccgcacgatccggctcacgaatgatcagctgaaatgcctcaacttgacgtacggtgaaaatgacttgaaatttagtgttgaccatggcaaagccattgtgaccagcaaattgtttgtctggcgctgggacgtccccatcgttatcagcgacattgacggtacgattacgaaaagtgatgcgctgggccacgtcctcgccatgatcggcaaagattggacccatctcggcgtcgctaagctgttcagtgagatctcgcgcaacggttacaatatcctgtacctgaccgcgcgctcggccggtcaggctgacagtacccgctcgtatctccgcagtattgagcagaacggtagcaagctcccgaacggccccgtcattctgagccccgatcggaccatggctgccctgcgccgggaggtgattctgaaaaagcccgaagtctttaaaatcgcttgcttgaacgatatccgctcgctctatttcgaagactcggataacgaagtggacacggaggaaaagagcacgccgtttttcgcgggctttggcaatcggatcaccgatgcgctcagctatcggacggtcggcatcccgagtagccgcatcttcacgattaacacggaaggcgaggtgcacatggagctgctcgagctcgccggttaccggagtagctatatccatatcaacgaactggtcgatcacttcttcccgccggtgagcctggactcggtcgatctgcgcacgaacacgagcatggtcccgggcagcccgccgaaccgcaccctggataactttgatagcgaaatcaccagtggccgcaagacgttgtttcgcggtaatcaggaggaaaaattcacggacgtcaacttttggcgcgatccgttggtggacatcgacaacctctcggatatcagtaacgatgattcggacaatattgatgaagacaccgatgtgagccaacagtcgaacatcagccgcaaccgcgctaactcggtcaagacggccaaggtgaccaaggctccgcagcggaatgtgtcgggcagtacgaataacaatgaagttctggctgcgagtagtgatgttgaaaatgccagtgacttggttagcagccactcgagtagcggctcgacccccaacaagtcgacgatgagtaagggtgatatcggcaaacaaatctatctggaactgggctcgcccttggcgagtcccaaactccggtatctggacgatatggatgatgaggactcgaactataatcgcaccaagagccgccgggctagtagcgccgctgctaccagcatcgacaaggagtttaaaaagctcagtgtgagtaaagctggcgctcccacccgcatcgttagcaagatcaacgtgtcgaatgatgtgcacagtttgggcaacagtgataccgaaagccggcgggaacagagcgtcaatgaaaccggtcgcaatcagttgccgcacaatagtatggatgataaggatttggattcgcgggtgagtgacgagttcgatgacgatgagtttgatgaagatgagtttgaggattag

SEQ ID NO: 9 - DNA, 6936 bp, Triticum aestivum
atgggatccacacatttgcccattgtcggccttaatgcctcgacaacaccatcgctatccactattcgcccggtaaattcagccggtgctgcattccaaccatctgccccttctagaacctccaagaagaaaagtcgtcgtgttcagtcattaagggatggaggcgatggaggcgtgtcagaccctaaccagtctattcgccaaggtcttgccggcatcattgacctcccaaaggagggcacatcagctccggaagtggatatttcacatgggtccgaagaacccaggggctcctaccaaatgaatgggatactgaatgaagcacataatgggaggcatgcttcgctgtctaaggttgtcgaattttgtatggcattgggcggcaaaacaccaattcacagtgtattagttgcgaacaatggaagggcagcagctaagttcatgcggagtgtccgaacatgggctaatgaaacatttgggtcagagaaggcaattcagttgatagctatggctactccagaagacatgaggataaatgcagagcacattagaattgctgatcaatttgttgaagtacccggtggaacaaacaataacaactatgcaaatgtccaactcatagtggagatagcagtgagaaccggtgtttctgctgtttggcctggttggggccatgcatctgagaatcctgaacttccagatgcactaaatgcaaacggaattgtttttcttgggccaccatcatcatcaatgaacgcactaggtgacaaggttggttcagctctcattgctcaagcagcaggggttccgactcttccttggggtggatcacaggtggaaattccattagaagtttgtttggactcgatacctgcggagatgtataggaaagcttgtgttagtactacggaggaagcacttgcgagttgtcagatgattgggtatccagccatgattaaagcatcatggggtggtggtggtaaagggatccgaaaggttaataacgacgatgatgtcagagcactgtttaagcaagtgcaaggtgaagttcctggctccccaatatttatcatgagacttgcatctcagagtcgacatcttgaagttcagttgctttgtgatcaatatggcaatgtagctgcgcttcacagtcgtgactgcagtgtgcaacggcgacaccaaaagattattgaggaaggaccagttactgttgctcctcgcgagacagtgaaagagctagagcaagcagcaaggaggcttgctaaggctgtgggttatgttggtgctgctactgttgaatatctctacagcatggagactggtgaatactattttctggaacttaatccacggttgcaggttgagcatccagtcaccgagtggatagctgaagtaaacttgcctgcagctcaagttgcagttggaatgggtatacccctttggcaggttccagagatcagacgtttctatggaatggacaatggaggaggctatgacatttggagggaaacagcagctcttgctactccatttaacttcgatgaagtggattctcaatggccaaagggtcattgtgtagcagttaggataaccagtgaggatccagatgacggattcaagcctaccggtggaaaagtaaaggagatcagttttaaaagcaagccaaatgtttgggcctatttctctgttaagtccggtggaggcattcatgaatttgctgattctcagtttggacatgtttttgcatatggagtgtctagagcagcagcaataaccaacatgtctcttgcgctaaaagagattcaaattcgtggagaaattcattcaaatgttgattacacagttgatctcttgaatgcctcagacttcaaagaaaacaggattcatactggctggctggataacagaatagcaatgcgagtccaagctgagagacctccgtggtatatttcagtggttggaggagctctatataaaacaataacgagcaacacagacactgtttctgaatatgttagctatctcgtcaagggtcagattccaccgaagcatatatcccttgtccattcaactgtttctttgaatatagaggaaagcaaatatacaattgaaactataaggagcggacagggtagctacagattgcgaatgaatggatcagttattgaagcaaatgtccaaacattatgtgatggtggacttttaatgcagttggatggaaacagccatgtaatttatgctgaagaagaggccggtggtacacggcttctaattgatggaaagacatacttgttacagaatgatcacgatccttcaaggttattagctgagacaccctgcaaacttcttcgtttcttggttgccgatggtgctcatgttgaagctgatgtaccatatgcggaagttgaggttatgaagatgtgcatgcccctcttgtcacctgctgctggtgtcattaatgttttgttgtctgagggccagcctatgcaggctggtgatcttatagcaagacttgatcttgatgacccttctgctgtgaagagagctgagccatttaacggatctttcccagaaatgagccttcctattgctgcttctggccaagttcacaaaagatgtgccacaagcttgaatgctgctcggatggtccttgcaggatatgatcacccgatcaacaaagttgtacaagatctggtatcctgtctagatgctcctgagcttcctttcctacaatgggaagagcttatgtctgttttagcaactagacttccaaggcttcttaagagcgagttggagggtaaatacagtgaatataagttaaatgttggccatgggaagagcaaggatttcccttccaagatgctaagagagataatcgaggaaaatcttgcacatggttctgagaaggaaattgctacaaatgagaggcttgttgagcctcttatgagcctactgaagtcatatgagggtggcagagaaagccatgcacactttattgtgaagtcccttttcgaggactatctctcggttgaggaactattcagtgatggcattcagtctgatgtgattgaacgcctgcgccaacaacatagtaaagatctccagaaggttgtagacattgtgttgtctcaccagggtgtgagaaacaaaactaagctgatactaacactcatggagaaactggtctatccaaaccctgctgtctacaaggatcagttgactcgcttttcctccctcaatcacaaaagatattataagttggcccttaaagctagcgagcttcttgaacaaaccaagcttagtgagctccgcacaagcattgcaaggagcctttcagaacttgagatgtttactgaagaaaggacggccattagtgagatcatgggagatttagtgactgccccactgccagttgaagatgcactggtttctttgtttgattgtagtgatcaaactcttcagcagagggtgatcgagacgtacatatctcgattataccagcctcatcttgtcaaggatagtatccagctgaaatatcaggaatctggtgttattgctttatgggaattcgctgaagcgcattcagagaagagattgggtgctatggttattgtgaagtcgttagaatctgtatcagcagcaattggagctgcactaaagggtacatcacgctatgcaagctctgagggtaacataatgcatattgctttattgggtgctgataatcaaatgcatggaactgaagacagtggtgataacgatcaagctcaagtcaggatagacaaactttctgcgacactggaacaaaatactgtcacagctgatctccgtgctgctggtgtgaaggttattagttgcattgttcaaagggatggagcactcatgcctatgcgccataccttcctcttgtcggatgaaaagctttgttatggggaagagccggttctccggcatgtggagcctcctctttctgctcttcttgagttgggtaagttgaaagtgaaaggatacaatgaggtgaagtatacaccgtcacgtgatcgtcagtggaacatatacacacttagaaatacagagaaccccaaaatgttgcacagggtgtttttccgaactcttgtcaggcaacccggtgcttccaacaaattcacatcaggcaacatcagtgatgttgaagtgggaggagctgaggaatctctttcatttacatcgagcagcatattaagatcgctgatgactgctatagaagagttggagcttcacgcgattaggacaggtcactctcatatgtttttgtgcatattgaaagagcgaaagcttcttgatcttgttcccgtttcagggaacaaagttgtggatattggccaagatgaagctactgcatgcttgcttctgaaagaaatggctctacagatacatgaacttgtgggtgcaaggatgcatcatctttctgtatgccaatgggaggtgaaacttaagttggacagcgatgggcctgccagtggtacctggagagttgtaacaaccaatgttactagtcacacctgcactgtggatatctaccgtgaggttgaagatacagaatcacagaaactagtataccactctgctccatcgtcatctggtcctttgcatggcgttgcactgaatactccatatcagcctttgagtgttattgatctgaaacgttgctccgctagaaacaacagaactacatactgctatgattttccgttggcatttgaaactgcagtgcagaagtcatggtctaacatttctagtgacaataaccgatgttatgttaaagcaacggagctggtgtttgctcacaagaatgggtcatggggcactcctgtaattcctatggagcgtcctgctgggctcaatgacattggtatggtagcttggatcttggacatgtccactcctgaatatcccaatggcaggcagattgttgtcatcgcaaatgatattacttttagagctggatcgtttggtccaagggaagatgcattttttgaaactgttaccaacctagcttgtgagaggaggcttcctctcatctacttggcagcaaactctggtgctcggatcggcatagcagatgaagtaaaatcttgcttccgtgttggatggtctgatgatggcagccctgaacgtgggtttcaatatatttatctgactgaagaagaccatgctcgtattagcgcttctgttatagcgcacaagatgcagcttgataatggtgaaattaggtgggttattgattctgttgtagggaaggaggatgggctaggtgtggagaacatacatggaagtgctgctattgccagtgcctattctagggcctatgaggagacatttacgcttacatttgtgactggaaggactgttggaataggagcatatcttgctcgacttggcatacggtgcattcagcgtactgaccagcccattatcctaactgggttttctgccttgaacaagcttcttggccgggaagtgtacagctcccacatgcagttgggtggccccaaaattatggcgacaaacggtgttgtccatctgacagtttcagatgaccttgaaggtgtatctaatatattgaggtggctcagctatgttcctgccaacattggtggacctcttcctattacaaaatctttggacccacctgacagacccgttgcttacatccctgagaatacatgcgatcctcgtgctgccatcagtggcattgatgatagccaagggaaatggttggggggcatgttcgacaaagacagttttgtggagacatttgaaggatgggcgaagtcagttgttactggcagagcgaaactcggagggattccggtgggtgttatagctgtggagacacagactatgatgcagctcatccctgctgatccaggccagcttgattcccatgagcgatctgttcctcgtgctgggcaagtctggtttccagattcagctactaagacagcgcaggcaatgctggacttcaaccgtgaaggattacctctgttcatccttgctaactggagaggcttctctggtggacaaagagatctttttgaaggaatccttcaggctgggtcaacaattgttgagaaccttagggcatacaatcagcctgcctttgtatatatccccaaggctgcagagctacgtggaggggcttgggtcgtgattgatagcaagataaatccagatcgcattgagttctatgctgagaggactgcaaagggcaatgttctcgaacctcaagggttgatcgagatcaagttcaggtcagaggaactccaagagtgcatgggtaggcttgatccagaattgataaatctgaaggcaaagctccagggagtaaagcatgaaaatggaagtctacctgagtcagaatcccttcagaagagcatagaagcccggaagaaacagttgttgcctttgtatactcaaattgcggtacggttcgctgaattgcatgacacttcccttagaatggctgctaagggtgtgattaagaaggttgtagactgggaagattctaggtcgttcttctacaagagattacggaggaggatatccgaggatgttcttgcgaaggaaattagaggtgtaagtggcaagcagttttctcaccaatcggcaatcgagctgatccagaaatggtacttggcctctaagggagctgaaacaggaagcactgaatgggatgatgacgatgcttttgttgcctggagggaaaaccctgaaaactaccaggagtatatcaaagaacccagggctcaaagggtatctcagttgctctcagatgttgcagactccagtccagatctagaagccttgccacagggtctttctatgctactagagaagatggatcctgcaaagagggaaattgttgaagactttgaaataaaccttgtaaagtaa

SEQ ID NO: 10 - DNA, 996 bp, Synechococcus PCC7942
atgtcagaggctcaaacgcccctgacagtaccgaagaagtttcttggtgctccaggaggcttcaaccccaccgtcgcactcttcttggcaggttatacctgcgcggcgctctcagttttggggtactggtgctggagttggccccactggctatctttccttctgagtgtcacagccttacatttggtaggcaccgtcattcacgatgcctctcataatgtggctcacgccagtcgcattctgaatgcgattttgggacatggcagtgcactattgctgggctttacttttccggtgtttacgcgggttcacctgcaacatcacgcccacgtcaacgatcccaagaacgatcccgaccacatcgtttccacctttgggccgctgtggttgatcgcaccgcgcttcttctatcacgagatctatttcttccagcgccgcctttggaagaaatttgaattactcgaatggttcctcagtcgcgctgtggtcatcggcatctttgcctgcggcgtcaagtttggcttcctgggcttcctgatgaactactggctggctccagccttggtcgttggcattgccctaggactcttcttcgactatttaccccaccgccccttccaagagcgcaaccgctggcgcaatgcacgggtctatcccggtcaggtgatgaacatcctgatcatgggtcagaactatcacctgatccatcacctctggccatcgatcccctggtatctctaccgaccggcctaccacgctaccaagccgttgttggacctacgccagtcgccgcaaacgctcgggattctctccagcaaaaaagatttctggaactttatctacgacgttttcatcggcatccgcattcaccaatcgcacgaggctgagccgcagagctccgtcgttcctgaaacgaagtcgagtgaatcagccgttctcgcaaaagctccgatgtctgccacagaagactctcgtgagccagccttgacgaagtag

SEQ ID NO: 11 - DNA, 486 bp, Brevundimonas sp. SD212
atggcctggctgacgtggatcgcgctgttcctgaccgcctttttgggcatggaggcgttcgcctggatcatgcaccgctatgtgatgcacggtttcctgtggtcctggcaccgcagccatcatgagccgcacgatcaccccctggagaagaacgacctgttcgccgtggtcttcgccgccccggccatcgtcatggtggccgtgggtctgcacctgtggccctgggccctgccggtcggcctggggatcacggcctatgggatggtctatttcttcttccacgacggcctggtgcaccggcggttcccgacgggcttttccgggcggtccggcttctggacgcggcgcatccaggcgcaccgtctgcatcacgccgtgcgcacgcgcgaaggctgcgtctccttcggctttctgtgggtgcggtcggcgcgggcgctgaaggccgaactggctcagaagcggggctcttccagcagcggcgcctga

SEQ ID NO: 12 - DNA, 735 bp, Brevundimonas sp. SD212
atgaccgccgccgtcgccgagccccgcatcgtcccgcgccagacctggatcggtctgaccctggcgggaatgatcgtggcgggatgggggagcctgcacgtctacggcgtctattttcaccgctggggcacctccagtctggtgatcgtcccggcgatcgtagcggtccagacctggttgtcggtcggccttttcatcgtcgcccatgacgccatgcacggctccctggcgccgggacggccgcggctgaacgccgcagtcggccggctgaccctggggctctatgcgggcttccgcttcgatcggctgaagacggcgcaccacgcccaccacgccgcgcccggcacggccgacgacccggacttttacgccccggcgccccgcgccttccttccctggttcctgaacttctttcgcacctatttcggctggcgcgagatggcggtcctgaccgccctggtcctgatcgccctcttcggcctgggggcgcggccggccaatctcctgaccttctgggccgcgccggccctgctttcagcgcttcagctcttcaccttcggcacctggctgccgcaccgccacaccgaccagccgttcgccgacgcccaccacgcccgcagcagcggctacggccccgttctttccctgctcacctgcttccacttcggccgccaccacgaacaccacctcaccccctggcggccctggtggcgtttgtggcgcggcgagtcttga

SEQ ID NO: 13 - DNA, 23 bp, Artificial Sequence
  primer to A. plantensis genome outside of homology arm
actactaatgtggctttccaggg

SEQ ID NO: 14 - DNA, 22 bp, Artificial Sequence
  primer to A. plantensis outside of the homology arm
gtaaattagcgcgatgggtttg

SEQ ID NO: 15 - DNA, 21 bp, Artificial Sequence
  primer to homology arm upstream of pilA gene
gttggagcaatggcacgagtc

SEQ ID NO: 16 - DNA, 23 bp, Artificial Sequence
  primer to upstream end of aadA gene
atgacgccaactacctctgatag

SEQ ID NO: 17 - DNA, 22 bp, Artificial Sequence
  primer to downstream end of aadA gene
gtatcagcccgtcatacttgaa

SEQ ID NO: 18 - DNA, 22 bp, Artificial Sequence
  primer to pilA gene
gacggtggtttcaccttaatcg

SEQ ID NO: 19 - DNA, 22 bp, Artificial Sequence
  primer to pilA gene
tgctgtagtacctacccagacc

SEQ ID NO: 20 - DNA, 20 bp, Artificial Sequence
  primer
cataccctgctgtgtggcaa

SEQ ID NO: 21 - DNA, 21 bp, Artificial Sequence
  primer
cgggtgatatctttggtggtg

SEQ ID NO: 22 - DNA, 22 bp, Artificial Sequence
  primer
gtacaaatgtacggccagcaac

SEQ ID NO: 23 - DNA, 528 bp, Artificial Sequence
  codon-optomized Pantoea ananatis beta-carotene 3,3'-hydroxylase (crtZ)
atgctgtggatttggaacgcgctgatcgtgtttgtcacagtcatcgggatggaagttattgccgccttggcacacaaatacatcatgcacggctggggctggggatggcatctgtctcaccacgaaccccgcaaaggcgctttcgaagtcaatgatctgtatgctgtcgtgtttgcagccctgagcattttgctcatctacctgggctcgaccggtatgtggccgttgcaatggattggtgccggcatgaccgcctacggtctgctgtatttcatggtgcacgatggcctggtccatcaacggtggccttttcggtatattccccgaaagggctacctgaagcgcctatatatggcccatcgaatgcatcacgcagtccgggggaaggaagggtgtgtgagttttgggtttctatatgctcccccgttgtcgaaactgcaagcaaccctgcgtgagcgtcatggcgctcgcgctggggcggcgcgggacgcgcaagggggcgaagatgaaccggcatcggggaaataa

SEQ ID NO: 24 - DNA, 720 bp, Artificial Sequence
  codon-optomized Brevundimonas sp. SD212 beta-carotene 4,4'-ketolase (crtW)
atgacggctgcggtcgctgagccgcgaatcgtgcctcgtcaaacctggatcgggctcacacttgcagggatgattgtggcaggctgggggagtcttcacgtctatggagtctactttcatcgctgggggacaagtagcctcgttattgtgccagcaatcgtggctgtccagacctggctcagtgtgggcctattcattgtcgcacacgacgctatgcacgggtcgctggcgccgggtcggcctcgcctaaacgcagccgtaggcagactcaccttagggctctatgccggtttccgatttgatcgccttaaaacggcccaccacgcacatcacgccgcccccggtactgccgatgaccctgatttctacgccccagcaccgcgagcgtttttgccttggttcctcaacttctttcgcacttactttggctggcgtgagatggctgttctgacagctttagtcctaatagccttgtttggtttgggtgcccggccggcaaatcttctcacgttctgggcagctccggcgctgttaagtgctctacagctattcacttttggcacgtggctgccgcaccgccacactgatcagccttttgcggacgcccaccatgctcggtcttccggttacggcccggtgctcagcctgcttacctgttttcactttggtcggcaccacgaacaccatctgacaccgtggcgcccctggtggcggctatgg

SEQ ID NO: 25 - DNA, 489 bp, Athrospira plantensis
atgaaaacccccctaaccgaagcagtttctatcgctgattcccaaggtcgtttcctaagcagcaccgaaatccaagtagcttttggccgttttcgtcaagccaaagctggtctggaagctgctaaagctttgacctctaaagctgatagtctgatcagtggtgctgcccaagcagtgtacaacaagttcccctacaccacccaaatgcagggacctaactacgcggcagaccaacgcggtaaggacaaatgtgctcgtgacataggctactacctgcggatggtaacttattgcctgattgctggtggaactggccccatggatgagtacctgattgccggtattgatgaaatcaaccggactttcgagctttctccaagctggtacattgaagccctgaaatacatcaaagctaaccacggtttgtctggtgacgctgctgttgaagctaactcctacctcgactacgcgatcaacgccctgagctag

SEQ ID NO: 26 - DNA, 519 bp, Athroisma gracile
atgtttgatgccttcaccaaggtggtttctcaagctgatactcgcggcgaaatgctgagtacagctcaaatcgatgctctgagccaaatggttgctgaaagcaacaaacgtttggattctgttaaccgcattaccagcaacgcttccaccattgtttccaacgctgctcgttctttgttcgcagagcaaccccaactgattgctcccggtggaaacgcctacaccagccgtcgtatggctgcttgcttgcgtgacatggaaatcatcctgcgctatgtaacctacgctgtgtttgctggcgatgcaagtgttctcgaagatcgttgcttgaacggtttgcgtgaaacttacctggctttgggaactcccggttcttccgttgctgtcggtgttggcaaaatgaaagaagctgctctggcgatcgttaacgatcccgcaggtatcactcctggtgattgtagcgctttggcttcagaaatcgctggttactttgaccgtgctgctgcagcagtttcctaa

SEQ ID NO: 27 - DNA, 1406 bp, Athrospira plantensis
ttgaaggggtgagaaggaaggcgaatgttgatttatgaagtttgattaacatttgtatcaaaatataaaattcttctcataaaccctgtacaatcttttaagatttcggaaagtgttctaggatactgaagaaatgaaccacggggcaattgttaaaagcctttgtcgatggttcgccccggaaggggtcttaggaggtgacaccgatggattgattgtcgtgatcattcatggtgtgtccaatcccaactcaactctaagcaagtcaacaagtaggagataaatccatgtttgatgccttcaccaaggtggtttctcaagctgatactcgcggcgaaatgctgagtacagctcaaatcgatgctctgagccaaatggttgctgaaagcaacaaacgtttggattctgttaaccgcattaccagcaacgcttccaccattgtttccaacgctgctcgttctttgttcgcagagcaaccccaactgattgctcccggtggaaacgcctacaccagccgtcgtatggctgcttgcttgcgtgacatggaaatcatcctgcgctatgtaacctacgctgtgtttgctggcgatgcaagtgttctcgaagatcgttgcttgaacggtttgcgtgaaacttacctggctttgggaactcccggttcttccgttgctgtcggtgttggcaaaatgaaagaagctgctctggcgatcgttaacgatcccgcaggtatcactcctggtgattgtagcgctttggcttcagaaatcgctggttactttgaccgtgctgctgcagcagtttcctaatcaagcagatccatagcatataacaattgaaacagtttagctgaagtctaagtgactggacttctgtttgttacctaattttttgtaaaccaatcgggagataactcgagaatgaaaacccccctaaccgaagcagtttctatcgctgattcccaaggtcgtttcctaagcagcaccgaaatccaagtagcttttggccgttttcgtcaagccaaagctggtctggaagctgctaaagctttgacctctaaagctgatagtctgatcagtggtgctgcccaagcagtgtacaacaagttcccctacaccacccaaatgcagggacctaactacgcggcagaccaacgcggtaaggacaaatgtgctcgtgacataggctactacctgcggatggtaacttattgcctgattgctggtggaactggccccatggatgagtacctgattgccggtattgatgaaatcaaccggactttcgagctttctccaagctggtacattgaagccctgaaatacatcaaagctaaccacggtttgtctggtgacgctgctgttgaagctaactcctacctcgactacgcgatcaacgccctgagctag